European Patent Application EP 4 298 924 A1, published January 3, 2024. Title: Composition for preventing, ameliorating or treating disease caused by nitration of protein comprising peptide with tyrosine at the terminal as effective component. Applicant: INDUSTRY-ACADEMIC COOPERATION FOUNDATION GYEONGSANG NATIONAL UNIVERSITY. The sequence listing filed with the application follows.

SEQUENCE LISTING (8 sequences)

SEQ ID NO: 1 - DNA, 23 bp, Artificial Sequence
  primer
tcgcagcagcacatcaacaagag

SEQ ID NO: 2 - DNA, 23 bp, Artificial Sequence
  primer
ggtgctcatgtcctcatcctgga

SEQ ID NO: 3 - DNA, 20 bp, Artificial Sequence
  primer
ccaattcatcttgaaatcac

SEQ ID NO: 4 - DNA, 20 bp, Artificial Sequence
  primer
ggaatgtccacaaactgata

SEQ ID NO: 5 - DNA, 20 bp, Artificial Sequence
  primer
acctttgaatgtgaagttga

SEQ ID NO: 6 - DNA, 20 bp, Artificial Sequence
  primer
ctacagaagtgcttgaggtg

SEQ ID NO: 7 - DNA, 21 bp, Artificial Sequence
  primer
gtggcaaagtggagattgttg

SEQ ID NO: 8 - DNA, 21 bp, Artificial Sequence
  primer
ttgactgtgccgttgaatttg